European Patent Application EP 4 170 032 A1, published April 26, 2023. Title: METHOD FOR DETERMINING DISEASES CAUSED BY OR ASSOCIATED WITH SYNAPTIC DYSFUNCTION. Applicant: AlzMed, Inc. The sequence listing filed with the application follows.

SEQUENCE LISTING (2 sequences)

SEQ ID NO: 1 - protein, 695 aa, Homo sapiens
MAGVSFSGHRLELLAAYEEVIREESAADWALYTYEDGSDDLKLAASGEGGLQELSGHFENQKVMYGFCSVKDSQAALPKYVLINWVGEDVPDARKCACASHVAKVAEFFQGVDVIVNASSVEDIDAGAIGQRLSNGLARLSSPVLHRLRLREDENAEPVGTTYQKTDAAVEMKRINREQFWEQAKKEEELRKEEERKKALDERLRFEQERMEQERQEQEERERRYREREQQIEEHRRKQQTLEAEEAKRRLKEQSIFGDHRDEEEETHMKKSESEVEEAAAIIAQRPDNPREFFKQQERVASASAGSCDVPSPFNHRPGRPYCPFIKASDSGPSSSSSSSSSPPRTPFPYITCHRTPNLSSSLPCSHLDSHRRMAPTPIPTRSPSDSSTASTPVAEQIERALDEVTSSQPPPLPPPPPPAQETQEPSPILDSEETRAAAPQAWAGPMEEPPQAQAPPRGPGSPAEDLMFMESAEQAVLAAPVEPATADATEIHDAADTIETDTATADTTVANNVPPAATSLIDLWPGNGEGASTLQGEPRAPTPPSGTEVTLAEVPLLDEVAPEPLLPAGEGCATLLNFDELPEPPATFCDPEEVEGEPLAAPQTPTLPSALEELEQEQEPEPHLLTNGETTQKEGTQASEGYFSQSQEEEFAQSEELCAKAPPPVFYNKPPEIDITCWDADPVPEEEEGFEGGD

SEQ ID NO: 2 - protein, 46 aa, Homo sapiens
RPYCPFIKASDSGPSSSSSSSSSPPRTPFPYITCHRTPNLSSSLPC